European Patent Specification EP 3 750 550 B1, published March 1, 2023. Title: Composition for preventing or treating osteoporosis. Applicant: PENS Co., LTD. KIM, HONG SIK. The sequence listing filed with the application follows.

SEQUENCE LISTING (12 sequences)

SEQ ID NO: 1 - DNA, 21 bp, Artificial Sequence
  GAPDH Primer F
atggaaatcccatcaccatct

SEQ ID NO: 2 - DNA, 18 bp, Artificial Sequence
  GAPDH Primer R
cgccccacttgattttgg

SEQ ID NO: 3 - DNA, 20 bp, Artificial Sequence
  ALP Primer F
ccgctttaaccagtgcaaca

SEQ ID NO: 4 - DNA, 20 bp, Artificial Sequence
  ALP Primer R
cccgattcatcacggagatg

SEQ ID NO: 5 - DNA, 18 bp, Artificial Sequence
  Osteocalcin Primer F
caggagggcagcgaggta

SEQ ID NO: 6 - DNA, 19 bp, Artificial Sequence
  Osteocalcin Primer R
gctcccagccattgataca

SEQ ID NO: 7 - DNA, 19 bp, Artificial Sequence
  NFATC-1 Primer F
tggcctcccgcttatctct

SEQ ID NO: 8 - DNA, 20 bp, Artificial Sequence
  NFATC-1 Primer R
ggataacgcaggcgaattgt

SEQ ID NO: 9 - DNA, 24 bp, Artificial Sequence
  Cathepsin K Primer F
gataatgtgaaccatgcagtgttg

SEQ ID NO: 10 - DNA, 20 bp, Artificial Sequence
  Cathepsin K Primer R
ccagtgcttgcttcccttct

SEQ ID NO: 11 - DNA, 19 bp, Artificial Sequence
  MMP-9 Primer F
acgccacgcattttcaaaa

SEQ ID NO: 12 - DNA, 18 bp, Artificial Sequence
  MMP-9 Primer R
ggcccattccctccacat